European Patent Specification EP 3 838 916 B1, published December 6, 2023. Title: Vaccine for preventing canine Toxoplasma gondii infection and preparation method thereof. Applicant: Hou Feng 2, 1. The sequence listing filed with the application follows.

SEQUENCE LISTING (3 sequences)

SEQ ID NO: 1 - DNA, 489 bp, Artificial sequence
atggaaaacgcgggcgtgcgcaaagcgtatatggatattgatattgatggcgaacatgcgggccgcattattctggaactgcgcgaagatattgcgaaaaaaaccgtgaaaaactttattggcctgtttgataaatataaaggcagcgtgtttcatcgcattattccggattttatgattcagggcggcgattttgaaaaccataacggcaccggcggccatagcatttatggccgccgctttgatgatgaaaactttgatctgaaacatgaacgcggcgtgattagcatggcgaacgcgggcccgaacaccaacggcagccagttttttattaccaccgtgaaaaccgaatggctggatgcgcgccatgtggtgtttggcaaaattaccaccgaaagctggccgaccgtgcaggcgattgaagcgctgggcggcagcggcggccgcccgagcaaagtggcgaaaattaccgatattggcaaaaaagaa

SEQ ID NO: 2 - protein, 163 aa, Artificial sequence
MENAGVRKAYMDIDIDGEHAGRIILELREDIAKKTVKNFIGLFDKYKGSVFHRIIPDFMIQGGDFENHNGTGGHSIYGRRFDDENFDLKHERGVISMANAGPNTNGSQFFITTVKTEWLDARHVVFGKITTESWPTVQAIEALGGSGGRPSKVAKITDIGKKE

SEQ ID NO: 3 - protein, 6 aa, Artificial sequence-label
HHHHHH